European Patent Specification EP 3 538 665 B1, published January 3, 2024. Title: PROTEASE SENSOR MOLECULES. Applicant: Commonwealth Scientific and Industrial Research Organisation. The sequence listing filed with the application follows.

SEQUENCE LISTING (123 sequences)

SEQ ID NO: 1 - protein, 4 aa, Artificial Sequence
  protease sensor molecule
KQKQ

SEQ ID NO: 2 - protein, 4 aa, Artificial Sequence
  Protease sensor molecule
KQSF

SEQ ID NO: 3 - protein, 4 aa, Artificial Sequence
  Protease sensor molecule
KQFM

SEQ ID NO: 4 - protein, 4 aa, Artificial Sequence
  Protease sensor molecule
KQKK

SEQ ID NO: 5 - protein, 4 aa, Artificial Sequence
  Protease sensor molecule
KQKN

SEQ ID NO: 6 - protein, 4 aa, Artificial Sequence
  Protease sensor molecule
KQNQ

SEQ ID NO: 7 - protein, 4 aa, Artificial Sequence
  Protease sensor molecule
KQNT

SEQ ID NO: 8 - protein, 4 aa, Artificial Sequence
  Protease sensor molecule
KQEI

SEQ ID NO: 9 - protein, 4 aa, Artificial Sequence
  Protease sensor molecule
SFSF

SEQ ID NO: 10 - protein, 4 aa, Artificial Sequence
  Protease sensor molecule
SFFM

SEQ ID NO: 11 - protein, 4 aa, Artificial Sequence
  Protease sensor molecule
SFKK

SEQ ID NO: 12 - protein, 4 aa, Artificial Sequence
  Protease sensor molecule
SFKN

SEQ ID NO: 13 - protein, 4 aa, Artificial Sequence
  Protease sensor molecule
SFNQ

SEQ ID NO: 14 - protein, 4 aa, Artificial Sequence
  Protease sensor molecule
SFNT

SEQ ID NO: 15 - protein, 4 aa, Artificial Sequence
  Protease sensor molecule
SFEI

SEQ ID NO: 16 - protein, 4 aa, Artificial Sequence
  Protease sensor molecule
FMFM

SEQ ID NO: 17 - protein, 4 aa, Artificial Sequence
  Protease sensor molecule
FMKK

SEQ ID NO: 18 - protein, 4 aa, Artificial Sequence
  Protease sensor molecule
FMKN

SEQ ID NO: 19 - protein, 4 aa, Artificial Sequence
  Protease sensor molecule
FMNQ

SEQ ID NO: 20 - protein, 4 aa, Artificial Sequence
  Protease sensor molecule
FMNT

SEQ ID NO: 21 - protein, 4 aa, Artificial Sequence
  Protease sensor molecule
FMEI

SEQ ID NO: 22 - protein, 4 aa, Artificial Sequence
  Protease sensor molecule
KKKK

SEQ ID NO: 23 - protein, 4 aa, Artificial Sequence
  Protease sensor molecule
KKKN

SEQ ID NO: 24 - protein, 4 aa, Artificial Sequence
  Protease sensor molecule
KKNQ

SEQ ID NO: 25 - protein, 4 aa, Artificial Sequence
  Protease sensor molecule
KKNT

SEQ ID NO: 26 - protein, 4 aa, Artificial Sequence
  Protease sensor molecule
KKEI

SEQ ID NO: 27 - protein, 4 aa, Artificial Sequence
  Protease sensor molecule
KNKN

SEQ ID NO: 28 - protein, 4 aa, Artificial Sequence
  Protease sensor molecule
KNNQ

SEQ ID NO: 29 - protein, 4 aa, Artificial Sequence
  Protease sensor molecule
KNNT

SEQ ID NO: 30 - protein, 4 aa, Artificial Sequence
  Protease sensor molecule
KNEI

SEQ ID NO: 31 - protein, 4 aa, Artificial Sequence
  Protease sensor molecule
KNFM

SEQ ID NO: 32 - protein, 4 aa, Artificial Sequence
  Protease sensor molecule
KNKK

SEQ ID NO: 33 - protein, 4 aa, Artificial Sequence
  Protease sensor molecule
NQNQ

SEQ ID NO: 34 - protein, 4 aa, Artificial Sequence
  Protease sensor molecule
NTNT

SEQ ID NO: 35 - protein, 4 aa, Artificial Sequence
  Protease sensor molecule
NTEI

SEQ ID NO: 36 - protein, 4 aa, Artificial Sequence
  Protease sensor molecule
EIEI

SEQ ID NO: 37 - protein, 3 aa, Artificial Sequence
  Protease sensor molecule
SFM

SEQ ID NO: 38 - protein, 7 aa, Artificial Sequence
  Protease sensor molecule
SFMKKNQ

SEQ ID NO: 39 - protein, 7 aa, Artificial Sequence
  Protease sensor molecule
KKNQSFM

SEQ ID NO: 40 - protein, 7 aa, Artificial Sequence
  Protease sensor molecule
  X (4)..(5): X can be any amino acid
SKMXXPP

SEQ ID NO: 41 - protein, 12 aa, Artificial Sequence
  Protease sensor molecule
  X (3)..(5): X can be any amino acid
  X (9)..(10): X can be any amino acid
PPXXXSKMXXPP

SEQ ID NO: 42 - protein, 11 aa, Artificial Sequence
  Protease sensor molecule
  X (3)..(4): X can be any amino acid
  X (8)..(9): X can be any amino acid
PPXXSKMXXPP

SEQ ID NO: 43 - protein, 10 aa, Artificial Sequence
  Protease sensor molecule
  X (3)..(3): X can be any amino acid
  X (7)..(8): X can be any amino acid
PPXSKMXXPP

SEQ ID NO: 44 - protein, 8 aa, Artificial Sequence
  Protease sensor molecule
PPVKQPPP

SEQ ID NO: 45 - protein, 11 aa, Artificial Sequence
  Protease sensor molecule
SFMKKNQNTEI

SEQ ID NO: 46 - protein, 11 aa, Artificial Sequence
  Protease sensor molecule
SFMNTKKNQEI

SEQ ID NO: 47 - protein, 11 aa, Artificial Sequence
  Protease sensor molecule
SFMQNTEIKKN

SEQ ID NO: 48 - protein, 11 aa, Artificial Sequence
  Protease sensor molecule
SFMNQKKNTEI

SEQ ID NO: 49 - protein, 11 aa, Artificial Sequence
  Protease sensor molecule
SFMNQNTKKEI

SEQ ID NO: 50 - protein, 11 aa, Artificial Sequence
  Protease sensor molecule
SFMNQNTEIKK

SEQ ID NO: 51 - protein, 11 aa, Artificial Sequence
  Protease sensor molecule
KKNQSFMNTEI

SEQ ID NO: 52 - protein, 11 aa, Artificial Sequence
  Protease sensor molecule
KKNQNTSFMEI

SEQ ID NO: 53 - protein, 11 aa, Artificial Sequence
  Protease sensor molecule
KKNQNTEISFM

SEQ ID NO: 54 - protein, 11 aa, Artificial Sequence
  Protease sensor molecule
KKSFMNQNTEI

SEQ ID NO: 55 - protein, 11 aa, Artificial Sequence
  Protease sensor molecule
KKNQSFMEINT

SEQ ID NO: 56 - protein, 11 aa, Artificial Sequence
  Protease sensor molecule
KKNQEISFMNT

SEQ ID NO: 57 - protein, 9 aa, Artificial Sequence
  Protease sensor molecule
SFMNQNTEI

SEQ ID NO: 58 - protein, 9 aa, Artificial Sequence
  Protease sensor molecule
NQSFMNTEI

SEQ ID NO: 59 - protein, 9 aa, Artificial Sequence
  Protease sensor molecule
NQNTSFMEI

SEQ ID NO: 60 - protein, 9 aa, Artificial Sequence
  Protease sensor molecule
NQNTEISFM

SEQ ID NO: 61 - protein, 9 aa, Artificial Sequence
  Protease sensor molecule
SFMNTNQEI

SEQ ID NO: 62 - protein, 9 aa, Artificial Sequence
  Protease sensor molecule
SFMNTEINQ

SEQ ID NO: 63 - protein, 9 aa, Artificial Sequence
  Protease sensor molecule
SFMNQEINT

SEQ ID NO: 64 - protein, 9 aa, Artificial Sequence
  Protease sensor molecule
NQSFMEINT

SEQ ID NO: 65 - protein, 9 aa, Artificial Sequence
  Protease sensor molecule
NQEISFMNT

SEQ ID NO: 66 - protein, 9 aa, Artificial Sequence
  Protease sensor molecule
SFMEINQNT

SEQ ID NO: 67 - protein, 9 aa, Artificial Sequence
  Protease sensor molecule
EISFMNTNQ

SEQ ID NO: 68 - protein, 9 aa, Artificial Sequence
  Protease sensor molecule
EINTSFMNQ

SEQ ID NO: 69 - protein, 9 aa, Artificial Sequence
  Protease sensor molecule
EINTNQSFM

SEQ ID NO: 70 - protein, 7 aa, Artificial Sequence
  Protease sensor molecule
LSFMAIP

SEQ ID NO: 71 - protein, 8 aa, Artificial Sequence
  Protease sensor molecule
LFMSFAIP

SEQ ID NO: 72 - protein, 18 aa, Artificial Sequence
  Protease sensor molecule
LQGSFMKKNQNTEIGSFE

SEQ ID NO: 73 - protein, 16 aa, Artificial Sequence
  Protease sensor molecule
LQGSFMNQNTEIGSFE

SEQ ID NO: 74 - protein, 15 aa, Artificial Sequence
  Protease sensor molecule
LQGSLSFMAIPGSFE

SEQ ID NO: 75 - protein, 4 aa, Artificial Sequence
  Protease sensor molecule
KQQQ

SEQ ID NO: 76 - protein, 4 aa, Artificial Sequence
  Protease sensor molecule
SFQQ

SEQ ID NO: 77 - protein, 4 aa, Artificial Sequence
  Protease sensor molecule
FMQQ

SEQ ID NO: 78 - protein, 4 aa, Artificial Sequence
  Protease sensor molecule
KKQQ

SEQ ID NO: 79 - protein, 4 aa, Artificial Sequence
  Protease sensor molecule
KNQQ

SEQ ID NO: 80 - protein, 4 aa, Artificial Sequence
  Protease sensor molecule
NQQQ

SEQ ID NO: 81 - protein, 4 aa, Artificial Sequence
  Protease sensor molecule
NTQQ

SEQ ID NO: 82 - protein, 4 aa, Artificial Sequence
  Protease sensor molecule
EIQQ

SEQ ID NO: 83 - protein, 4 aa, Artificial Sequence
  Protease sensor molecule
QQQQ

SEQ ID NO: 84 - protein, 4 aa, Artificial Sequence
  Protease sensor molecule
QQKQ

SEQ ID NO: 85 - protein, 4 aa, Artificial Sequence
  Protease sensor molecule
QQSF

SEQ ID NO: 86 - protein, 4 aa, Artificial Sequence
  Protease sensor molecule
QQFM

SEQ ID NO: 87 - protein, 4 aa, Artificial Sequence
  Protease sensor molecule
QQKK

SEQ ID NO: 88 - protein, 4 aa, Artificial Sequence
  Protease sensor molecule
QQKN

SEQ ID NO: 89 - protein, 4 aa, Artificial Sequence
  Protease sensor molecule
QQNQ

SEQ ID NO: 90 - protein, 4 aa, Artificial Sequence
  Protease sensor molecule
QQNT

SEQ ID NO: 91 - protein, 4 aa, Artificial Sequence
  Protease sensor molecule
QQEI

SEQ ID NO: 92 - protein, 3 aa, Artificial Sequence
  Protease sensor molecule
KQQ

SEQ ID NO: 93 - protein, 12 aa, Artificial Sequence
  Protease sensor molecule
GSPPLQQPPPGS

SEQ ID NO: 94 - protein, 16 aa, Artificial Sequence
  Protease sensor molecule
GGSGGSLKQQGGSGGS

SEQ ID NO: 95 - protein, 3 aa, Artificial Sequence
  Protease sensor molecule
LQG

SEQ ID NO: 96 - protein, 4 aa, Artificial Sequence
  Protease sensor molecule
GSFE

SEQ ID NO: 97 - protein, 6 aa, Artificial Sequence
  Protease sensor molecule
GSSGGS

SEQ ID NO: 98 - protein, 5 aa, Artificial Sequence
  Protease sensor molecule
GSPPL

SEQ ID NO: 99 - protein, 5 aa, Artificial Sequence
  Protease sensor molecule
PPPGS

SEQ ID NO: 100 - protein, 6 aa, Artificial Sequence
  Protease Sensor Molecule
GGSGGS

SEQ ID NO: 101 - protein, 7 aa, Artificial Sequence
  Protease Sensor Molecule
GGSGGSL

SEQ ID NO: 102 - DNA, 1713 bp, Artificial Sequence
  Protease Sensor Molecule
gaattcatggtgagcaagggcgaggagctgttcaccggggtggtgcccatcctggtcgagctggacggcgacgtaaacggccacaagttcagcgtgtccggcgagggcgagggcgatgccacctacggcaagctgaccctgaagttcatctgcaccaccggcaagctgcccgtgccctggcccaccctcgtgaccaccctgagctacggcgtgcagtgcttcagccgctaccccgaccacatgaagcagcacgacttcttcaagtccgccatgcccgaaggctacgtccaggagcgcaccatcttcttcaaggacgacggcaactacaagacccgcgccgaggtgaagttcgagggcgacaccctggtgaaccgcatcgagctgaagggcatcgacttcaaggaggacggcaacatcctggggcacaagctggagtacaactacaacagccacaacgtctatatcatggccgacaagcagaagaacggcatcaaggtgaacttcaagatccgccacaacatcgaggacggcagcgtgcagctcgccgaccactaccagcagaacacccccatcggcgacggccccgtgctgctgcccgacaaccactacctgagcacccagtccgccctgagcaaagaccccaacgagaagcgcgatcacatggtcctgctggagttcgtgaccgccgccgggatcactctcggcatggacgagctgtacaagctgcagggttcctttatgaaccagaacactgaaatcggaagcttcgaaatggcttccaaggtgtacgaccccgagcaacgcaaacgcatgatcactgggcctcagtggtgggctcgctgcaagcaaatgaacgtgctggactccttcatcaactactatgattccgagaagcacgccgagaacgccgtgatttttctgcatggtaacgctgcctccagctacctgtggaggcacgtcgtgcctcacatcgagcccgtggctagatgcatcatccctgatctgatcggaatgggtaagtccggcaagagcgggaatggctcatatcgcctcctggatcactacaagtacctcaccgcttggttcgagctgctgaaccttccaaagaaaatcatctttgtgggccacgactggggggctgctctggcctttcactactcctacgagcaccaagacaagatcaaggccatcgtccatgctgagagtgtcgtggacgtgatcgagtcctgggacgagtggcctgacatcgaggaggatatcgccctgatcaagagcgaagagggcgagaaaatggtgcttgagaataacttcttcgtcgagaccgtgctcccaagcaagatcatgcggaaactggagcctgaggagttcgctgcctacctggagccattcaaggagaagggcgaggttagacggcctaccctctcctggcctcgcgagatccctctcgttaagggaggcaagcccgacgtcgtccagattgtccgcaactacaacgcctaccttcgggccagcgacgatctgcctaagatgttcatcgagtccgaccctgggttcttttccaacgctattgtcgagggagctaagaagttccctaacaccgagttcgtgaaggtgaagggcctccacttcagccaggaggacgctccagatgaaatgggtaagtacatcaagagcttcgtggagcgcgtgctgaagaacgagcagtaactcgag

SEQ ID NO: 103 - DNA, 1713 bp, Artificial Sequence; identical to SEQ ID NO: 102
  Protease Sensor Molecule

SEQ ID NO: 104 - DNA, 1710 bp, Artificial Sequence
  Protease Sensor Molecule
gaattcatggtgagcaagggcgaggagctgttcaccggggtggtgcccatcctggtcgagctggacggcgacgtaaacggccacaagttcagcgtgtccggcgagggcgagggcgatgccacctacggcaagctgaccctgaagttcatctgcaccaccggcaagctgcccgtgccctggcccaccctcgtgaccaccctgagctacggcgtgcagtgcttcagccgctaccccgaccacatgaagcagcacgacttcttcaagtccgccatgcccgaaggctacgtccaggagcgcaccatcttcttcaaggacgacggcaactacaagacccgcgccgaggtgaagttcgagggcgacaccctggtgaaccgcatcgagctgaagggcatcgacttcaaggaggacggcaacatcctggggcacaagctggagtacaactacaacagccacaacgtctatatcatggccgacaagcagaagaacggcatcaaggtgaacttcaagatccgccacaacatcgaggacggcagcgtgcagctcgccgaccactaccagcagaacacccccatcggcgacggccccgtgctgctgcccgacaaccactacctgagcacccagtccgccctgagcaaagaccccaacgagaagcgcgatcacatggtcctgctggagttcgtgaccgccgccgggatcactctcggcatggacgagctgtacaagctgcagggctctttaagctttatggccatccctggttccttcgaaatggcttccaaggtgtacgaccccgagcaacgcaaacgcatgatcactgggcctcagtggtgggctcgctgcaagcaaatgaacgtgctggactccttcatcaactactatgattccgagaagcacgccgagaacgccgtgatttttctgcatggtaacgctgcctccagctacctgtggaggcacgtcgtgcctcacatcgagcccgtggctagatgcatcatccctgatctgatcggaatgggtaagtccggcaagagcgggaatggctcatatcgcctcctggatcactacaagtacctcaccgcttggttcgagctgctgaaccttccaaagaaaatcatctttgtgggccacgactggggggctgctctggcctttcactactcctacgagcaccaagacaagatcaaggccatcgtccatgctgagagtgtcgtggacgtgatcgagtcctgggacgagtggcctgacatcgaggaggatatcgccctgatcaagagcgaagagggcgagaaaatggtgcttgagaataacttcttcgtcgagaccgtgctcccaagcaagatcatgcggaaactggagcctgaggagttcgctgcctacctggagccattcaaggagaagggcgaggttagacggcctaccctctcctggcctcgcgagatccctctcgttaagggaggcaagcccgacgtcgtccagattgtccgcaactacaacgcctaccttcgggccagcgacgatctgcctaagatgttcatcgagtccgaccctgggttcttttccaacgctattgtcgagggagctaagaagttccctaacaccgagttcgtgaaggtgaagggcctccacttcagccaggaggacgctccagatgaaatgggtaagtacatcaagagcttcgtggagcgcgtgctgaagaacgagcagtaactcgag

SEQ ID NO: 105 - protein, 568 aa, Artificial Sequence
  Protease Sensor Molecule
MVSKGEELFTGVVPILVELDGDVNGHKFSVSGEGEGDATYGKLTLKFICTTGKLPVPWPTLVTTLSYGVQCFSRYPDHMKQHDFFKSAMPEGYVQERTIFFKDDGNYKTRAEVKFEGDTLVNRIELKGIDFKEDGNILGHKLEYNYNSHNVYIMADKQKNGIKVNFKIRHNIEDGSVQLADHYQQNTPIGDGPVLLPDNHYLSTQSALSKDPNEKRDHMVLLEFVTAAGITLGMDELYKLQGSFMKKNQNTEIGSFEMASKVYDPEQRKRMITGPQWWARCKQMNVLDSFINYYDSEKHAENAVIFLHGNAASSYLWRHVVPHIEPVARCIIPDLIGMGKSGKSGNGSYRLLDHYKYLTAWFELLNLPKKIIFVGHDWGAALAFHYSYEHQDKIKAIVHAESVVDVIESWDEWPDIEEDIALIKSEEGEKMVLENNFFVETVLPSKIMRKLEPEEFAAYLEPFKEKGEVRRPTLSWPREIPLVKGGKPDVVQIVRNYNAYLRASDDLPKMFIESDPGFFSNAIVEGAKKFPNTEFVKVKGLHFSQEDAPDEMGKYIKSFVERVLKNEQ

SEQ ID NO: 106 - protein, 566 aa, Artificial Sequence
  Protease Sensor Molecule
MVSKGEELFTGVVPILVELDGDVNGHKFSVSGEGEGDATYGKLTLKFICTTGKLPVPWPTLVTTLSYGVQCFSRYPDHMKQHDFFKSAMPEGYVQERTIFFKDDGNYKTRAEVKFEGDTLVNRIELKGIDFKEDGNILGHKLEYNYNSHNVYIMADKQKNGIKVNFKIRHNIEDGSVQLADHYQQNTPIGDGPVLLPDNHYLSTQSALSKDPNEKRDHMVLLEFVTAAGITLGMDELYKLQGSFMNQNTEIGSFEMASKVYDPEQRKRMITGPQWWARCKQMNVLDSFINYYDSEKHAENAVIFLHGNAASSYLWRHVVPHIEPVARCIIPDLIGMGKSGKSGNGSYRLLDHYKYLTAWFELLNLPKKIIFVGHDWGAALAFHYSYEHQDKIKAIVHAESVVDVIESWDEWPDIEEDIALIKSEEGEKMVLENNFFVETVLPSKIMRKLEPEEFAAYLEPFKEKGEVRRPTLSWPREIPLVKGGKPDVVQIVRNYNAYLRASDDLPKMFIESDPGFFSNAIVEGAKKFPNTEFVKVKGLHFSQEDAPDEMGKYIKSFVERVLKNEQ

SEQ ID NO: 107 - protein, 565 aa, Artificial Sequence
  Protease Sensor Molecule
MVSKGEELFTGVVPILVELDGDVNGHKFSVSGEGEGDATYGKLTLKFICTTGKLPVPWPTLVTTLSYGVQCFSRYPDHMKQHDFFKSAMPEGYVQERTIFFKDDGNYKTRAEVKFEGDTLVNRIELKGIDFKEDGNILGHKLEYNYNSHNVYIMADKQKNGIKVNFKIRHNIEDGSVQLADHYQQNTPIGDGPVLLPDNHYLSTQSALSKDPNEKRDHMVLLEFVTAAGITLGMDELYKLQGSLSFMAIPGSFEMASKVYDPEQRKRMITGPQWWARCKQMNVLDSFINYYDSEKHAENAVIFLHGNAASSYLWRHVVPHIEPVARCIIPDLIGMGKSGKSGNGSYRLLDHYKYLTAWFELLNLPKKIIFVGHDWGAALAFHYSYEHQDKIKAIVHAESVVDVIESWDEWPDIEEDIALIKSEEGEKMVLENNFFVETVLPSKIMRKLEPEEFAAYLEPFKEKGEVRRPTLSWPREIPLVKGGKPDVVQIVRNYNAYLRASDDLPKMFIESDPGFFSNAIVEGAKKFPNTEFVKVKGLHFSQEDAPDEMGKYIKSFVERVLKNEQ

SEQ ID NO: 108 - DNA, 1710 bp, Artificial Sequence
  Protease Sensor Molecule
gaattcatggtgagcaagggcgaggagctgttcaccggggtggtgcccatcctggtcgagctggacggcgacgtaaacggccacaagttcagcgtgtccggcgagggcgagggcgatgccacctacggcaagctgaccctgaagttcatctgcaccaccggcaagctgcccgtgccctggcccaccctcgtgaccaccctgagctacggcgtgcagtgcttcagccgctaccccgaccacatgaagcagcacgacttcttcaagtccgccatgcccgaaggctacgtccaggagcgcaccatcttcttcaaggacgacggcaactacaagacccgcgccgaggtgaagttcgagggcgacaccctggtgaaccgcatcgagctgaagggcatcgacttcaaggaggacggcaacatcctggggcacaagctggagtacaactacaacagccacaacgtctatatcatggccgacaagcagaagaacggcatcaaggtgaacttcaagatccgccacaacatcgaggacggcagcgtgcagctcgccgaccactaccagcagaacacccccatcggcgacggccccgtgctgctgcccgacaaccactacctgagcacccagtccgccctgagcaaagaccccaacgagaagcgcgatcacatggtcctgctggagttcgtgaccgccgccgggatcactctcggcatggacgagctgtacaagctgcagggttccaaaaagtataaagttaaggaaggatcacttcagatggcttccaaggtgtacgaccccgagcaacgcaaacgcatgatcactgggcctcagtggtgggctcgctgcaagcaaatgaacgtgctggactccttcatcaactactatgattccgagaagcacgccgagaacgccgtgatttttctgcatggtaacgctgcctccagctacctgtggaggcacgtcgtgcctcacatcgagcccgtggctagatgcatcatccctgatctgatcggaatgggtaagtccggcaagagcgggaatggctcatatcgcctcctggatcactacaagtacctcaccgcttggttcgagctgctgaaccttccaaagaaaatcatctttgtgggccacgactggggggctgctctggcctttcactactcctacgagcaccaagacaagatcaaggccatcgtccatgctgagagtgtcgtggacgtgatcgagtcctgggacgagtggcctgacatcgaggaggatatcgccctgatcaagagcgaagagggcgagaaaatggtgcttgagaataacttcttcgtcgagaccgtgctcccaagcaagatcatgcggaaactggagcctgaggagttcgctgcctacctggagccattcaaggagaagggcgaggttagacggcctaccctctcctggcctcgcgagatccctctcgttaagggaggcaagcccgacgtcgtccagattgtccgcaactacaacgcctaccttcgggccagcgacgatctgcctaagatgttcatcgagtccgaccctgggttcttttccaacgctattgtcgagggagctaagaagttccctaacaccgagttcgtgaaggtgaagggcctccacttcagccaggaggacgctccagatgaaatgggtaagtacatcaagagcttcgtggagcgcgtgctgaagaacgagcagtaactcgag

SEQ ID NO: 109 - protein, 565 aa, Artificial Sequence
  Protease Sensor Molecule
MVSKGEELFTGVVPILVELDGDVNGHKFSVSGEGEGDATYGKLTLKFICTTGKLPVPWPTLVTTLSYGVQCFSRYPDHMKQHDFFKSAMPEGYVQERTIFFKDDGNYKTRAEVKFEGDTLVNRIELKGIDFKEDGNILGHKLEYNYNSHNVYIMADKQKNGIKVNFKIRHNIEDGSVQLADHYQQNTPIGDGPVLLPDNHYLSTQSALSKDPNEKRDHMVLLEFVTAAGITLGMDELYKLQGSKKYKVKEGSLQMASKVYDPEQRKRMITGPQWWARCKQMNVLDSFINYYDSEKHAENAVIFLHGNAASSYLWRHVVPHIEPVARCIIPDLIGMGKSGKSGNGSYRLLDHYKYLTAWFELLNLPKKIIFVGHDWGAALAFHYSYEHQDKIKAIVHAESVVDVIESWDEWPDIEEDIALIKSEEGEKMVLENNFFVETVLPSKIMRKLEPEEFAAYLEPFKEKGEVRRPTLSWPREIPLVKGGKPDVVQIVRNYNAYLRASDDLPKMFIESDPGFFSNAIVEGAKKFPNTEFVKVKGLHFSQEDAPDEMGKYIKSFVERVLKNEQ

SEQ ID NO: 110 - protein, 11 aa, Artificial Sequence
  Protease sensor molecule
  X (3)..(6): X can be any amino acid
  Z (8)..(8): Z is is lysine, tyrosine, valine or glutamic acid
LQXXXXKZKLQ

SEQ ID NO: 111 - protein, 15 aa, Artificial Sequence
  Protease sensor molecule
LQGSKKYKVKEGSLQ

SEQ ID NO: 112 - protein, 16 aa, Artificial Sequence
  Protease sensor molecule
LQGSKQKQKQKQGSFE

SEQ ID NO: 113 - protein, 16 aa, Artificial Sequence
  Protease sensor molecule
LQGSPPLKQPPPGSFE

SEQ ID NO: 114 - protein, 16 aa, Artificial Sequence
  Protease sensor molecule
LQGSPPLQQPQPGSFE

SEQ ID NO: 115 - protein, 20 aa, Artificial Sequence
  Protease sensor molecule
LQGGSGGSLKQQGGSGGSFE

SEQ ID NO: 116 - DNA, 1701 bp, Artificial Sequence
  Nucleotide sequence encoding GFP2-Pflu-H1-RLuc2
atggtgagcaagggcgaggagctgttcaccggggtggtgcccatcctggtcgagctggacggcgacgtaaacggccacaagttcagcgtgtccggcgagggcgagggcgatgccacctacggcaagctgaccctgaagttcatctgcaccaccggcaagctgcccgtgccctggcccaccctcgtgaccaccctgagctacggcgtgcagtgcttcagccgctaccccgaccacatgaagcagcacgacttcttcaagtccgccatgcccgaaggctacgtccaggagcgcaccatcttcttcaaggacgacggcaactacaagacccgcgccgaggtgaagttcgagggcgacaccctggtgaaccgcatcgagctgaagggcatcgacttcaaggaggacggcaacatcctggggcacaagctggagtacaactacaacagccacaacgtctatatcatggccgacaagcagaagaacggcatcaaggtgaacttcaagatccgccacaacatcgaggacggcagcgtgcagctcgccgaccactaccagcagaacacccccatcggcgacggccccgtgctgctgcccgacaaccactacctgagcacccagtccgccctgagcaaagaccccaacgagaagcgcgatcacatggtcctgctggagttcgtgaccgccgccgggatcactctcggcatggacgagctgtacaagctgcagggaagtccaccgttgaaacaaccccctcctggctccttcgaaatggcttccaaggtgtacgaccccgagcaacgcaaacgcatgatcactgggcctcagtggtgggctcgctgcaagcaaatgaacgtgctggactccttcatcaactactatgattccgagaagcacgccgagaacgccgtgatttttctgcatggtaacgctgcctccagctacctgtggaggcacgtcgtgcctcacatcgagcccgtggctagatgcatcatccctgatctgatcggaatgggtaagtccggcaagagcgggaatggctcatatcgcctcctggatcactacaagtacctcaccgcttggttcgagctgctgaaccttccaaagaaaatcatctttgtgggccacgactggggggctgctctggcctttcactactcctacgagcaccaagacaagatcaaggccatcgtccatgctgagagtgtcgtggacgtgatcgagtcctgggacgagtggcctgacatcgaggaggatatcgccctgatcaagagcgaagagggcgagaaaatggtgcttgagaataacttcttcgtcgagaccgtgctcccaagcaagatcatgcggaaactggagcctgaggagttcgctgcctacctggagccattcaaggagaagggcgaggttagacggcctaccctctcctggcctcgcgagatccctctcgttaagggaggcaagcccgacgtcgtccagattgtccgcaactacaacgcctaccttcgggccagcgacgatctgcctaagatgttcatcgagtccgaccctgggttcttttccaacgctattgtcgagggagctaagaagttccctaacaccgagttcgtgaaggtgaagggcctccacttcagccaggaggacgctccagatgaaatgggtaagtacatcaagagcttcgtggagcgcgtgctgaagaacgagcagtaa

SEQ ID NO: 117 - DNA, 1707 bp, Artificial Sequence
  Nucleotide sequence encoding GFP2-Pflu-H2-RLuc2
atggtgagcaagggcgaggagctgttcaccggggtggtgcccatcctggtcgagctggacggcgacgtaaacggccacaagttcagcgtgtccggcgagggcgagggcgatgccacctacggcaagctgaccctgaagttcatctgcaccaccggcaagctgcccgtgccctggcccaccctcgtgaccaccctgagctacggcgtgcagtgcttcagccgctaccccgaccacatgaagcagcacgacttcttcaagtccgccatgcccgaaggctacgtccaggagcgcaccatcttcttcaaggacgacggcaactacaagacccgcgccgaggtgaagttcgagggcgacaccctggtgaaccgcatcgagctgaagggcatcgacttcaaggaggacggcaacatcctggggcacaagctggagtacaactacaacagccacaacgtctatatcatggccgacaagcagaagaacggcatcaaggtgaacttcaagatccgccacaacatcgaggacggcagcgtgcagctcgccgaccactaccagcagaacacccccatcggcgacggccccgtgctgctgcccgacaaccactacctgagcacccagtccgccctgagcaaagaccccaacgagaagcgcgatcacatggtcctgctggagttcgtgaccgccgccgggatcactctcggcatggacgagctgtacaagctgcagggatctccacccttacaacaaccgcaaccgggtagcttcgaaatggcttccaaggtgtacgaccccgagcaacgcaaacgcatgatcactgggcctcagtggtgggctcgctgcaagcaaatgaacgtgctggactccttcatcaactactatgattccgagaagcacgccgagaacgccgtgatttttctgcatggtaacgctgcctccagctacctgtggaggcacgtcgtgcctcacatcgagcccgtggctagatgcatcatccctgatctgatcggaatgggtaagtccggcaagagcgggaatggctcatatcgcctcctggatcactacaagtacctcaccgcttggttcgagctgctgaaccttccaaagaaaatcatctttgtgggccacgactggggggctgctctggcctttcactactcctacgagcaccaagacaagatcaaggccatcgtccatgctgagagtgtcgtggacgtgatcgagtcctgggacgagtggcctgacatcgaggaggatatcgccctgatcaagagcgaagagggcgagaaaatggtgcttgagaataacttcttcgtcgagaccgtgctcccaagcaagatcatgcggaaactggagcctgaggagttcgctgcctacctggagccattcaaggagaagggcgaggttagacggcctaccctctcctggcctcgcgagatccctctcgttaagggaggcaagcccgacgtcgtccagattgtccgcaactacaacgcctaccttcgggccagcgacgatctgcctaagatgttcatcgagtccgaccctgggttcttttccaacgctattgtcgagggagctaagaagttccctaacaccgagttcgtgaaggtgaagggcctccacttcagccaggaggacgctccagatgaaatgggtaagtacatcaagagcttcgtggagcgcgtgctgaagaacgagcagtaactcgag

SEQ ID NO: 118 - DNA, 1707 bp, Artificial Sequence
  Nucleotide sequence encoding GFP2-Pflu-H3-RLuc2
atggtgagcaagggcgaggagctgttcaccggggtggtgcccatcctggtcgagctggacggcgacgtaaacggccacaagttcagcgtgtccggcgagggcgagggcgatgccacctacggcaagctgaccctgaagttcatctgcaccaccggcaagctgcccgtgccctggcccaccctcgtgaccaccctgagctacggcgtgcagtgcttcagccgctaccccgaccacatgaagcagcacgacttcttcaagtccgccatgcccgaaggctacgtccaggagcgcaccatcttcttcaaggacgacggcaactacaagacccgcgccgaggtgaagttcgagggcgacaccctggtgaaccgcatcgagctgaagggcatcgacttcaaggaggacggcaacatcctggggcacaagctggagtacaactacaacagccacaacgtctatatcatggccgacaagcagaagaacggcatcaaggtgaacttcaagatccgccacaacatcgaggacggcagcgtgcagctcgccgaccactaccagcagaacacccccatcggcgacggccccgtgctgctgcccgacaaccactacctgagcacccagtccgccctgagcaaagaccccaacgagaagcgcgatcacatggtcctgctggagttcgtgaccgccgccgggatcactctcggcatggacgagctgtacaagctgcaggggtctaaacaaaaacagaagcaaaagcaaggatcattcgaaatggcttccaaggtgtacgaccccgagcaacgcaaacgcatgatcactgggcctcagtggtgggctcgctgcaagcaaatgaacgtgctggactccttcatcaactactatgattccgagaagcacgccgagaacgccgtgatttttctgcatggtaacgctgcctccagctacctgtggaggcacgtcgtgcctcacatcgagcccgtggctagatgcatcatccctgatctgatcggaatgggtaagtccggcaagagcgggaatggctcatatcgcctcctggatcactacaagtacctcaccgcttggttcgagctgctgaaccttccaaagaaaatcatctttgtgggccacgactggggggctgctctggcctttcactactcctacgagcaccaagacaagatcaaggccatcgtccatgctgagagtgtcgtggacgtgatcgagtcctgggacgagtggcctgacatcgaggaggatatcgccctgatcaagagcgaagagggcgagaaaatggtgcttgagaataacttcttcgtcgagaccgtgctcccaagcaagatcatgcggaaactggagcctgaggagttcgctgcctacctggagccattcaaggagaagggcgaggttagacggcctaccctctcctggcctcgcgagatccctctcgttaagggaggcaagcccgacgtcgtccagattgtccgcaactacaacgcctaccttcgggccagcgacgatctgcctaagatgttcatcgagtccgaccctgggttcttttccaacgctattgtcgagggagctaagaagttccctaacaccgagttcgtgaaggtgaagggcctccacttcagccaggaggacgctccagatgaaatgggtaagtacatcaagagcttcgtggagcgcgtgctgaagaacgagcagtaactcgag

SEQ ID NO: 119 - DNA, 1713 bp, Artificial Sequence
  Nucleotide sequence encoding GFP2-Pflu-H4-RLuc2
atggtgagcaagggcgaggagctgttcaccggggtggtgcccatcctggtcgagctggacggcgacgtaaacggccacaagttcagcgtgtccggcgagggcgagggcgatgccacctacggcaagctgaccctgaagttcatctgcaccaccggcaagctgcccgtgccctggcccaccctcgtgaccaccctgagctacggcgtgcagtgcttcagccgctaccccgaccacatgaagcagcacgacttcttcaagtccgccatgcccgaaggctacgtccaggagcgcaccatcttcttcaaggacgacggcaactacaagacccgcgccgaggtgaagttcgagggcgacaccctggtgaaccgcatcgagctgaagggcatcgacttcaaggaggacggcaacatcctggggcacaagctggagtacaactacaacagccacaacgtctatatcatggccgacaagcagaagaacggcatcaaggtgaacttcaagatccgccacaacatcgaggacggcagcgtgcagctcgccgaccactaccagcagaacacccccatcggcgacggccccgtgctgctgcccgacaaccactacctgagcacccagtccgccctgagcaaagaccccaacgagaagcgcgatcacatggtcctgctggagttcgtgaccgccgccgggatcactctcggcatggacgagctgtacaagctgcaggggggaagcggtggtagtttgaaacagcagggcggatcaggagggtctttcgaaatggcttccaaggtgtacgaccccgagcaacgcaaacgcatgatcactgggcctcagtggtgggctcgctgcaagcaaatgaacgtgctggactccttcatcaactactatgattccgagaagcacgccgagaacgccgtgatttttctgcatggtaacgctgcctccagctacctgtggaggcacgtcgtgcctcacatcgagcccgtggctagatgcatcatccctgatctgatcggaatgggtaagtccggcaagagcgggaatggctcatatcgcctcctggatcactacaagtacctcaccgcttggttcgagctgctgaaccttccaaagaaaatcatctttgtgggccacgactggggggctgctctggcctttcactactcctacgagcaccaagacaagatcaaggccatcgtccatgctgagagtgtcgtggacgtgatcgagtcctgggacgagtggcctgacatcgaggaggatatcgccctgatcaagagcgaagagggcgagaaaatggtgcttgagaataacttcttcgtcgagaccgtgctcccaagcaagatcatgcggaaactggagcctgaggagttcgctgcctacctggagccattcaaggagaagggcgaggttagacggcctaccctctcctggcctcgcgagatccctctcgttaagggaggcaagcccgacgtcgtccagattgtccgcaactacaacgcctaccttcgggccagcgacgatctgcctaagatgttcatcgagtccgaccctgggttcttttccaacgctattgtcgagggagctaagaagttccctaacaccgagttcgtgaaggtgaagggcctccacttcagccaggaggacgctccagatgaaatgggtaagtacatcaagagcttcgtggagcgcgtgctgaagaacgagcagtaa

SEQ ID NO: 120 - protein, 566 aa, Artificial Sequence
  GFP2-Pflu-H1-RLuc2 fusion protein
MVSKGEELFTGVVPILVELDGDVNGHKFSVSGEGEGDATYGKLTLKFICTTGKLPVPWPTLVTTLSYGVQCFSRYPDHMKQHDFFKSAMPEGYVQERTIFFKDDGNYKTRAEVKFEGDTLVNRIELKGIDFKEDGNILGHKLEYNYNSHNVYIMADKQKNGIKVNFKIRHNIEDGSVQLADHYQQNTPIGDGPVLLPDNHYLSTQSALSKDPNEKRDHMVLLEFVTAAGITLGMDELYKLQGSPPLKQPPPGSFEMASKVYDPEQRKRMITGPQWWARCKQMNVLDSFINYYDSEKHAENAVIFLHGNAASSYLWRHVVPHIEPVARCIIPDLIGMGKSGKSGNGSYRLLDHYKYLTAWFELLNLPKKIIFVGHDWGAALAFHYSYEHQDKIKAIVHAESVVDVIESWDEWPDIEEDIALIKSEEGEKMVLENNFFVETVLPSKIMRKLEPEEFAAYLEPFKEKGEVRRPTLSWPREIPLVKGGKPDVVQIVRNYNAYLRASDDLPKMFIESDPGFFSNAIVEGAKKFPNTEFVKVKGLHFSQEDAPDEMGKYIKSFVERVLKNEQ

SEQ ID NO: 121 - protein, 567 aa, Artificial Sequence
  GFP2-Pflu-H2-RLuc2 fusion protein
MVSKGEELFTGVVPILVELDGDVNGHKFSVSGEGEGDATYGKLTLKFICTTGKLPVPWPTLVTTLSYGVQCFSRYPDHMKQHDFFKSAMPEGYVQERTIFFKDDGNYKTRAEVKFEGDTLVNRIELKGIDFKEDGNILGHKLEYNYNSHNVYIMADKQKNGIKVNFKIRHNIEDGSVQLADHYQQNTPIGDGPVLLPDNHYLSTQSALSKDPNEKRDHMVLLEFVTAAGITLGMDELYKLQGSPPLQQPQPGSFEMASKVYDPEQRKRMITGPQWWARCKQMNVLDSFINYYDSEKHAENAVIFLHGNAASSYLWRHVVPHIEPVARCIIPDLIGMGKSGKSGNGSYRLLDHYKYLTAWFELLNLPKKIIFVGHDWGAALAFHYSYEHQDKIKAIVHAESVVDVIESWDEWPDIEEDIALIKSEEGEKMVLENNFFVETVLPSKIMRKLEPEEFAAYLEPFKEKGEVRRPTLSWPREIPLVKGGKPDVVQIVRNYNAYLRASDDLPKMFIESDPGFFSNAIVEGAKKFPNTEFVKVKGLHFSQEDAPDEMGKYIKSFVERVLKNEQE

SEQ ID NO: 122 - protein, 566 aa, Artificial Sequence
  GFP2-Pflu-H3-RLuc2 fusion protein
MVSKGEELFTGVVPILVELDGDVNGHKFSVSGEGEGDATYGKLTLKFICTTGKLPVPWPTLVTTLSYGVQCFSRYPDHMKQHDFFKSAMPEGYVQERTIFFKDDGNYKTRAEVKFEGDTLVNRIELKGIDFKEDGNILGHKLEYNYNSHNVYIMADKQKNGIKVNFKIRHNIEDGSVQLADHYQQNTPIGDGPVLLPDNHYLSTQSALSKDPNEKRDHMVLLEFVTAAGITLGMDELYKLQGSKQKQKQKQGSFEMASKVYDPEQRKRMITGPQWWARCKQMNVLDSFINYYDSEKHAENAVIFLHGNAASSYLWRHVVPHIEPVARCIIPDLIGMGKSGKSGNGSYRLLDHYKYLTAWFELLNLPKKIIFVGHDWGAALAFHYSYEHQDKIKAIVHAESVVDVIESWDEWPDIEEDIALIKSEEGEKMVLENNFFVETVLPSKIMRKLEPEEFAAYLEPFKEKGEVRRPTLSWPREIPLVKGGKPDVVQIVRNYNAYLRASDDLPKMFIESDPGFFSNAIVEGAKKFPNTEFVKVKGLHFSQEDAPDEMGKYIKSFVERVLKNEQ

SEQ ID NO: 123 - protein, 570 aa, Artificial Sequence
  GFP2-Pflu-H4-RLuc2 fusion protein
MVSKGEELFTGVVPILVELDGDVNGHKFSVSGEGEGDATYGKLTLKFICTTGKLPVPWPTLVTTLSYGVQCFSRYPDHMKQHDFFKSAMPEGYVQERTIFFKDDGNYKTRAEVKFEGDTLVNRIELKGIDFKEDGNILGHKLEYNYNSHNVYIMADKQKNGIKVNFKIRHNIEDGSVQLADHYQQNTPIGDGPVLLPDNHYLSTQSALSKDPNEKRDHMVLLEFVTAAGITLGMDELYKLQGGSGGSLKQQGGSGGSFEMASKVYDPEQRKRMITGPQWWARCKQMNVLDSFINYYDSEKHAENAVIFLHGNAASSYLWRHVVPHIEPVARCIIPDLIGMGKSGKSGNGSYRLLDHYKYLTAWFELLNLPKKIIFVGHDWGAALAFHYSYEHQDKIKAIVHAESVVDVIESWDEWPDIEEDIALIKSEEGEKMVLENNFFVETVLPSKIMRKLEPEEFAAYLEPFKEKGEVRRPTLSWPREIPLVKGGKPDVVQIVRNYNAYLRASDDLPKMFIESDPGFFSNAIVEGAKKFPNTEFVKVKGLHFSQEDAPDEMGKYIKSFVERVLKNEQ